European Patent Application EP 4 356 972 A2, published April 24, 2024. Title: ANTI-ANNEXIN A2 MONOCLONAL ANTIBODIES. Applicant: Agency for Science, Technology and Research. Application EP. The sequence listing filed with the application follows.

SEQUENCE LISTING (30 sequences)

SEQ ID NO: 1 - protein, 116 aa, synthetic construct
  REGION 1..116: note = Isolated antibody
VQLQESGPDLVKPSRSLSLTCTVTGYSITSGYSWHWIRQFPGNKLEWMGYIHYSGSTKYNPSLKSRISITRDTSKNQFFLQLNSVTTEDAATYYCARGSNYGFDYWGQGTTLTVSS

SEQ ID NO: 2 - protein, 114 aa, synthetic construct
  REGION 1..114: note = Isolated antibody
DIELTQSPSSLAVSVGEKVTMSCKSSQSLLYSNDQKNYLAWYQQKPGQSPKLLIYWASIRESGVPDRFTGSGSGTDFTLTISSVKAEDLAVYYCQQYYIYPLTFGAGTKLEIKR

SEQ ID NO: 3 - DNA, 348 bp, synthetic construct
  misc_feature 1..348: note = Isolated antibody
  source 1..348: mol_type = other DNA
gtacagctgcaggagtcaggacctgacctggtgaaaccttctcggtcactttcactcacctgcactgtcactggctactccatcaccagtggttatagctggcactggatccggcagtttccaggaaacaaactggaatggatgggctacatacactacagtggtagcactaagtacaacccatctctcaaaagtcgaatctctatcactcgagacacatccaagaaccagttcttcctgcagttgaattctgtgactactgaggacgcagccacatattactgtgcaagggggagtaactacggatttgactactggggccaaggcaccactctcacagtctcctca

SEQ ID NO: 4 - DNA, 342 bp, synthetic construct
  misc_feature 1..342: note = Isolated antibody
  source 1..342: mol_type = other DNA
gacattgagctcacccagtctccatcctccctagctgtgtcagttggagagaaggttactatgagctgcaagtccagtcagagccttttatatagtaacgatcaaaagaactacttggcctggtaccaacagaaaccagggcagtctcctaaactgctgatttactgggcatctattagggaatctggggtccctgatcgcttcacaggcagtggatctgggacagatttcactctcaccatcagcagtgtgaaggctgaagacctggcagtttattactgtcagcaatattatatctatcctctcacgttcggtgctgggaccaagctggaaataaaacgg

SEQ ID NO: 5 - protein, 117 aa, synthetic construct
  REGION 1..117: note = Isolated antibody
QVKLQESGPDQVKPSQSLSLTCTVTVYSITSGYSWHWIRQFPGNKLEWMGYIHYSGSTKYNPSLKSRFSITRDTSKNQFFLQLNSVTTEDTATYYCARGTDNAVDYWGQGTTVTVSS

SEQ ID NO: 6 - protein, 114 aa, synthetic construct
  REGION 1..114: note = Isolated antibody
DIELTQSPSSLAVSVGEKVNMSCKSSQSLLYSSNQKNYLAWYQQKPGQSPKLLIYWASSRESGVPDRFTGSGSGTDFTLTISSVKAEDLAVYYCQQYYIYPLTFGAGTKLELKR

SEQ ID NO: 7 - DNA, 351 bp, synthetic construct
  misc_feature 1..351: note = Isolated antibody
  source 1..351: mol_type = other DNA
caggtgaaactgcaggagtcaggacctgaccaggtgaaaccctctcagtcactttcactcacctgcactgtcactgtctactccatcaccagtggttatagctggcactggatccggcagtttccaggaaacaaactggaatggatgggctacatacactacagtggtagtactaagtacaacccatctctcaaaagtcgattctctatcactcgagacacatccaagaaccagttcttcctgcagttgaattctgtgactactgaggacacagccacatattactgtgcaagagggaccgacaatgctgtggactactggggccaagggaccacggtcaccgtctcctca

SEQ ID NO: 8 - DNA, 342 bp, synthetic construct
  misc_feature 1..342: note = Isolated antibody
  source 1..342: mol_type = other DNA
gacattgagctcacccagtctccatcctccctagctgtgtcagttggagagaaggttaatatgagctgcaagtccagtcagagccttttatatagtagcaatcaaaagaactacttggcctggtaccagcagaaaccagggcagtctcctaaattgctgatttactgggcatccagtagggaatctggggtccctgatcgcttcacaggcagtggatctgggacagatttcactctcaccatcagcagtgtgaaggctgaagacctggcagtttattactgtcagcaatattatatctatcctctcacgttcggtgctgggaccaagctggagctgaaacgg

SEQ ID NO: 9 - protein, 11 aa, synthetic construct
  REGION 1..11: note = Isolated antibody
GYSITSGYSWH

SEQ ID NO: 10 - protein, 16 aa, synthetic construct
  REGION 1..16: note = Isolated antibody
YIHYSGSTKYNPSLKS

SEQ ID NO: 11 - protein, 8 aa, synthetic construct
  REGION 1..8: note = Isolated antibody
GSNYGFDY

SEQ ID NO: 12 - protein, 17 aa, synthetic construct
  REGION 1..17: note = Isolated antibody
KSSQSLLYSNDQKNYLA

SEQ ID NO: 13 - protein, 7 aa, synthetic construct
  REGION 1..7: note = Isolated antibody
WASIRES

SEQ ID NO: 14 - protein, 9 aa, synthetic construct
  REGION 1..9: note = Isolated antibody
QQYYIYPLT

SEQ ID NO: 15 - DNA, 32 bp, synthetic construct
  misc_feature 1..32: note = Isolated antibody
  source 1..32: mol_type = other DNA
gctactccatcaccagtggttatagctggcac

SEQ ID NO: 16 - DNA, 48 bp, synthetic construct
  misc_feature 1..48: note = Isolated antibody
  source 1..48: mol_type = other DNA
acatacactacagtggtagcactaagtacaacccatctctcaaaagtc

SEQ ID NO: 17 - DNA, 24 bp, synthetic construct
  misc_feature 1..24: note = Isolated antibody
  source 1..24: mol_type = other DNA
ggagtaactacggatttgactact

SEQ ID NO: 18 - DNA, 51 bp, synthetic construct
  misc_feature 1..51: note = Isolated antibody
  source 1..51: mol_type = other DNA
agtccagtcagagccttttatatagtaacgatcaaaagaactacttggcct

SEQ ID NO: 19 - DNA, 21 bp, synthetic construct
  misc_feature 1..21: note = Isolated antibody
  source 1..21: mol_type = other DNA
gggcatctattagggaatctg

SEQ ID NO: 20 - DNA, 27 bp, synthetic construct
  misc_feature 1..27: note = Isolated antibody
  source 1..27: mol_type = other DNA
agcaatattatatctatcctctcacgt

SEQ ID NO: 21 - protein, 11 aa, synthetic construct
  REGION 1..11: note = Isolated antibody
VYSITSGYSWH

SEQ ID NO: 22 - protein, 8 aa, synthetic construct
  REGION 1..8: note = Isolated antibody
GTDNAVDY

SEQ ID NO: 23 - protein, 17 aa, synthetic construct
  REGION 1..17: note = Isolated antibody
KSSQSLLYSSNQKNYLA

SEQ ID NO: 24 - protein, 7 aa, synthetic construct
  REGION 1..7: note = Isolated antibody
WASSRES

SEQ ID NO: 25 - DNA, 33 bp, synthetic construct
  misc_feature 1..33: note = Isolated antibody
  source 1..33: mol_type = other DNA
tctactccatcaccagtggttatagctggcact

SEQ ID NO: 26 - DNA, 48 bp, synthetic construct
  misc_feature 1..48: note = Isolated antibody
  source 1..48: mol_type = other DNA
acatacactacagtggtagtactaagtacaacccatctctcaaaagtc

SEQ ID NO: 27 - DNA, 24 bp, synthetic construct
  misc_feature 1..24: note = Isolated antibody
  source 1..24: mol_type = other DNA
ggaccgacaatgctgtggactact

SEQ ID NO: 28 - DNA, 51 bp, synthetic construct
  misc_feature 1..51: note = Isolated antibody
  source 1..51: mol_type = other DNA
agtccagtcagagccttttatatagtagcaatcaaaagaactacttggcct

SEQ ID NO: 29 - DNA, 21 bp, synthetic construct
  misc_feature 1..21: note = Isolated antibody
  source 1..21: mol_type = other DNA
gggcatccagtagggaatctg

SEQ ID NO: 30 - protein, 339 aa, synthetic construct
  REGION 1..339: note = Isolated antibody
MSTVHEILCKLSLEGDHSTPPSAYGSVKAYTNFDAERDALNIETAIKTKGVDEVTIVNILTNRSNAQRQDIAFAYQRRTKKELASALKSALSGHLETVILGLLKTPAQYDASELKASMKGLGTDEDSLIEIICSRTNQELQEINRVYKEMYKTDLEKDIISDTSGDFRKLMVALAKGRRAEDGSVIDYELIDQDARDLYDAGVKRKGTDVPKWISIMTERSVPHLQKVFDRYKSYSPYDMLESIRKEVKGDLENAFLNLVQCIQNKPLYFADRLYDSMKGKGTRDKVLIRIMVSRSEVDMLKIRSEFKRKYGKSLYYYIQQDTKGDYQKALLYLCGGDD